European Patent Application EP 4 494 651 A2, published January 22, 2025. Title: MODIFIED VIRUSES. Applicant: Mayo Foundation for Medical Education and Research. Application EP, filed April 4, 2018. The sequence listing filed with the application follows.

SEQUENCE LISTING (15 sequences)

SEQ ID NO: 1 - protein, 617 aa, measles virus
MSPQRDRINAFYKDNPHPKGSRIVINREHLMIDRPYVLLAVLFVMFLSLIGLLAIAGIRLHRAAIYTAEIHKSLSTNLDVTNSIEHQVKDVLTPLFKIIGDEVGLRTPQRFTDLVKLISDKIKFLNPDREYDFRDLTWCINPPERIKLDYDQYCADVAAEELMNALVNSTLLETRTTNQFLAVSKGNCSGPTTIRGQFSNMSLSLLDLYLGRGYNVSSIVTMTSQGMYGGTYLVEKPNLSSKRSELSQLSMYRVFEVGVIRNPGLGAPVFHMTNYLEQPVSNDLSNCMVALGELKLAALCHGEDSITIPYQGSGKGVSFQLVKLGVWKSPTDMQSWVPLSTDDPVIDRLYLSSHRGVIADNQAKWAVPTTRTDDKLRMETCFQQACKGKIQALCENPEWAPLKDNRIPSYGVLSVDLSLTVELKIKIASGFGPLITHGSGMDLYKSNHNNVYWLTIPPMKNLALGVINTLEWIPRFKVSPYLFTVPIKEAGEDCHAPTYLPAEVDGDVKLSSNLVILPGQDLQYVLATYDTSRVEHAVVYYVYSPSRSFSYFYPFRLPIKGVPIELQVECFTWDQKLWCRHFCVLADSESGGHITHSGMVGMGVSCTVTREDGTNRR

SEQ ID NO: 2 - DNA, 1854 bp, measles virus
  source 1..1854: mol_type = other DNA
atgtcaccgcaaagagaccggataaatgccttctacaaagataacccttatcccaagggaagtaggatagttattaacagagaacatcttatgattgacagaccctatattctgctggctgttctgttcgtcatgtttctgagcttgatcggattgctggcaattgcaggcattagacttcatcgggcagccatctacaccgcggagatccataaaagcctcagtaccaatctagatgtgactaactcaatcgagcatcaggtcaaggacgtgctgacaccactctttaaaatcatcggggatgaagtgggcctgagaacacctcagagattcactgacctagtgaaattcatctctgacaagattaaattccttaatccggatagggagtacgacttcagagatctcacttggtgcatcaacccgccagagaggatcaaactagattatgatcaatactgtgcagatgtggctgctgaagagctcatgaatgcattggtgaactcaactctactggagaccagaacaaccaatcagttcctagctgtctcaaagggaaactgctcagggcccactacaatcagaggtcaattctcaaacatgtcgctgtccttgttggacttgtacttaggtcgaggttacaatgtgtcatctatagtcactatgacatcccagggaatgtatgggggaacctacctagtggaaaagcctaatctgaacagcaaagggtcagagttgtcacaactgagcatgtaccgagtgtttgaagtaggtgttatcagaaacccgggtttgggggctccggtgttccatatgacaaactattttgagcaaccagtcagtaatggtctcggcaactgtatggtggctttgggggagctcaaactcgcagccctttgtcacggggacgattctatcacaattccctatcagggatcagggaaaggtgtcagcttccagctcgtcaagctgggtgtctggaaatccccaaccgacatgcaatcctgggtccccttatcaacggatgatccagtggtagacaggctttacctctcatctcacagaggtgtcatcgctgacaatcaagcaaaatgggctgtcccgacaacacgaacagatgacaagttgcgaatggagacatgcttccagcaggcgtgtaaaggtaaaatccaagcactctgcgagaatcccgagtgggtgccattgaaggataacaggattccttcatacggggtcctgtctgttgatctgagtctgacagttgagcttaaaatcaaaattgcttcgggattcgggccattgatcacacacggctcagggatggacctatacaaatccaaccgcaacaatgtgtattggctgactattccgccaatgagaaatctagccttaggcgtaatcaacacattggagtggataccgagattcaaggttagtcccaacctcttcactgtcccaattaaggaagcaggcgaggactgccatgccccaacatacctacctgcggaggtggacggtgatgtcaaactcagttccaacctggtgattctacctggtcaagatctccaatatgttttggcaacctacgatacctccagggttgagcatgctgtggtttattacgtttacagcccaagccgctcattttcttacttttatccttttaggttgcctataaagggggtcccaatcgaactacaagtggaatgcttcacatgggaccaaaaactctggtgccgtcacttctgtgtgcttgcggactcagaatccggcggacatatcactcactctgggatggtgggcatgggagtcagctgcacagctacccgggaagatggaaccaatcgcagataa

SEQ ID NO: 3 - protein, 617 aa, synthetic construct
  REGION 1..617: note = construct sequence
MSPQRDRINAFYKDNPHSKGSRIVINREHLMIDRPYVLLAVLFVMFLSLIGLLAIAGIRLHRAAIYTAEIHKSLSTNLDVTNSIEHQVKDVLTPLFKIIGDEVGLRTPQRFTDLVKFISDKIKFLNPDREYDFRDLTWCINPPERIKLNYDQYCADVAAEELMNALVNSTLLETRTTNQFLAVSKGNCPGPTTIRGQFSNMSLSLLDLYLSRGYNVSSIVTMTSQGMYGGTYLVGKPDLNSKGSELSQPSMYRVFEVGVIRNPGLGAPVFHMTNYFEQPISKDLSNCMVALGELKLAALCHRGDSITIPCRGSGKGVSFQLVKLGVWKSPTDMHSWVPLSTDDPVIDRLYLSSHRGVITDNQANWAVPTTRTDDKLQKETCFQQACKGKIQALCENLEWAPLKDSRIPSYGVLSVNLSLAAEPKIKIASGFGPLITHGSGMDLYKSNHNNVYWLTIPPMKNLALGVINTLEWIPRLKVSPYLFTVPIEEADEDCRAPTYLPAEVTGDVKLSSNLVILPGQDLQYVLATYDTSGVEHAVVYYVYSPGGSFSYVYPFRLPIKGTPIELQVECFTWAQRLWCRHFCVLADSESGGHLTHSGMVGMEVSCTVNREDEANRR

SEQ ID NO: 4 - protein, 553 aa, measles virus
MSIMGLKVNVSAIFMAVLLTLQTPTGQIHWGNLSKIGVVGIGSASYKVMTRSSHQSLVIKLMPNITLLNNCTRVEIAEYRRLLRTVLEPIRDALNAMTQNIRPVQSVASSRRHKRFAGVVLAGAALGVATAAQITAGIALHQSMLNSQAIDNLRASLETTNQAIETIRQAGQEMILAVQGVQDYINNELIPSMNQLSCDLIGQKLGLKLLRYYTEILSLFGPSLRDPISAEISIQALSYALGGDINKVLEKLGYSGGDLLGILESGGIKARITHVDTESYFIVLSIAYPTLSEIKGVIVHRLEGVSYNIGSQEWYTTVPKYVATQGYLISNFDESSCTFMPEGTVCSQNALYPMSPLLQECLRGYTKSCARTLVSGSFGNRFILSQGNLIANCASILCKCYTTGTIINQDPDKILTYIAADHCPVVEVNGVTIQVGSRRYPDAVYLHRIDLGPPISLERLDVGTNLGNAIAKLEDAKELLESSDQILRSMKGLSSTSIVYILIAVCLGGLIGIPALICCCRGRCNKKGEQVGMSRPGLKPDLTGTSKSYVRSL

SEQ ID NO: 5 - protein, 1653 aa, measles virus
ATGGGTCTCAAGGTGAACGTCTCTGCCGTATTCATGGCAGTACTGTTAACTCTCCAAACACCCGCCGGTCAAATTCATTGGGGCAATCTCTCTAAGATAGGGGTAGTAGGAATAGGAAGTGCAAGCTACAAAGTTATGACTCGTTCCAGCCATCAATCATTAGTCATAAAATTAATGCCCAATATAACTCTCCTCAATAACTGCACGAGGGTAGAGATTGCAGAATACAGGAGACTACTAAGAACAGTTTTGGAACCAATTAGGGATGCACTTAATGCAATGACCCAGAACATAAGGCCGGTTCAGAGCGTAGCTTCAAGTAGGAGACACAAGAGATTTGCGGGAGTAGTCCTGGCAGGTGCGGCCCTAGGTGTTGCCACAGCTGCTCAGATAACAGCCGGCATTGCACTTCACCGGTCCATGCTGAACTCTCAGGCCATCGACAATCTGAGAGCGAGCCTGGAAACTACTAATCAGGCAATTGAGGCAATCAGACAAGCAGGGCAGGAGATGATATTGGCTGTTCAGGGTGTCCAAGACTACATCAATAATGAGCTGATACCGTCTATGAACCAGCTATCTTGTGATCTAATCGGTCAGAAGCTCGGGCTCAAATTGCTTAGATACTATACAGAAATCCTGTCATTATTTGGCCCCAGCCTACGGGACCCCATATCTGCGGAGATATCTATCCAGGCTTTGAGTTATGCACTTGGAGGAGATATCAATAAGGTGTTAGAAAAGCTCGGATACAGTGGAGGCGATTTACTAGGCATCTTAGAGAGCAGAGGAATAAAGGCTCGGATAACTCACGTCGACACAGAGTCCTACTTCATAGTCCTCAGTATAGCCTATCCGACGCTGTCCGAGATTAAGGGGGTGATTGTCCACCGGCTAGAGGGGGTCTCGTACAACATAGGCTCTCAAGAGTGGTATACCACTGTGCCCAAGTATGTTGCAACCCAAGGGTACCTTATCTCGAATTTTGATGAGTCATCATGTACTTTCATGCCAGAGGGGACTGTGTGCAGCCAAAATGCCTTGTACCCGATGAGTCCTCTGCTCCAAGAATGCCTCCGGGGGTCCACCAAGTCCTGTGCTCGTACACTCGTATCCGGGTCTTTTGGGAACCGGTTCATTTTATCACAAGGGAACCTAATAGCCAATTGTGCATCAATTCTTTGTAAGTGTTACACAACAGGTACGATTATTAATCAAGACCCTGACAAGATCCTAACATACATTGCTGCCGATCGCTGCCCGGTAGTCGAGGTGAACGGCGTGACCATCCAAGTCGGGAGCAGGAGGTATCCAGACGCTGTGTACTTGCACAGAATTGACCTCGGTCCTCCCATATCATTGGAGAGGTTGGACGTAGGGACAAATCTGGGGAATGCAATTGCCAAATTGGAGGATGCCAAGGAATTGTTGGAATCATCGGACCAGATATTGAGAAGTATGAAAGGTTTATCGAGCACTAGCATAGTCTACATCCTGATTGCAGTGTGTCTTGGAGGGTTGATAGGGATCCCCACTTTAATATGTTGCTGCAGGGGGCGTTGTAACAAAAAGGGAGAACAAGTTGGTATGTCAAGACCAGGCCTAAAGCCTGACCTTACAGGAACATCAAAATCCTATGTAAGATCGCTTTGA

SEQ ID NO: 6 - protein, 662 aa, canine distemper virus
MHNKNPKKSKPLPHTRQDPLQQHSTRSAETKTSQGQHSTTSAQRSTYHGPRTSDRSVHYIMNRTRSCKQTSHRSDNIPPHRDHEGIIHHTPESVTQGASSWFKRRQSNATNAGSQYTWLVLWCIGIASLLLCSKAQIHWNNLSTIGIIGTDSVHYKIMTRPSHQYLVIKLMPNVSLIDNCTKAELGEYEKLLNSVLEPINQALTLMTNNVKPLQSVGSGRRQRRFAGVVLAGAALGVATAAQITAGIALHQSNLNAQAIQSLRTSLEQSNKAIEEIREATQETVIAVQGVQDYVNNELVPAMQHMSCELVGQRLGLKLLRYYTELLSIFGPSLRDPISAEISIQALSYALGGEIHKILEKLGYSGNDMIAILESRGIKTKITHVDLPGKLIILSISYPTLSEVKGVIVHRLEAVSYNIGSQEWYTTVPKYVATNGYLISNFDESSCVFVSESAICSQNSLYPMSPILQQCIRGDTSSCARTLVSGTMGNKFILSKGNIVANCASILCKCYSTSTIINQSPDKLLTFIASDTCPLVEIDGVTIQVGGRQYPDMVYESKVALGPAISLERLDVGTNLGNALKKLDDAKVLIDSSNQILETVKRSSFNFGSLLSVPILICTALALLLLIYCCKRRYRQTFKHNTKVDPTFKPDLTGTSKSYVRSL

SEQ ID NO: 7 - protein, 662 aa, canine distemper virus
MHNKIPKRSKPLPHTRQDPLQQHSTRFGETTTSQGRHSTTSAQRSTHHGPRTSDRPVHHTMNRTRSCKQTSHRSDNILPHRDHKGIIHHTPESVTQGASSWFKRRQFNATNAGSQCTWLVLWCIGIASLFLCSKAQIHWNNLSTIGIIGTDSVHYKIMTRPSHQYLVIKLMPNVSLIDNCTKAELGEYEKLLNSVLEPINQALTLMTNNVKPLQSVGSGRRQRRFAGVVLAGAALGVATAAQITAGIALHQSNLNAQAIQSLRTSLEQSNKAIEEIREATQETVIAVQGVQDYVNNELVPAMQHMSCELVGQRLGLKLLRYYTELLSIFGPSLRDPISAEISIQALSYALGGEIHKILEKLGYSGNDMIAILESRGIKTKITHVDLPGKLIILSISYPTLSEVKGVIVHRLETVSYNIGSQEWYTTVPKYVATNGYLISNFDESSCVFFSESAICSQNSLYPMSPILQQCIRGDTSSCARTLVSGTMGNKFILSKGNIVANCASILCKCYSTSTIINQSPDKLLTFIASDTCPLVEIDGVTIQVGGRQYPDMVYESKVALGPAISLERLDVGTNLGNALKKLDDAKVLIDSSNQILETVKRSSFNFGSLLSIPILICTALVLLLLIYCCNRRYRQTFKHNTKVDPTFKPDLTGTSKSYVRSL

SEQ ID NO: 8 - protein, 604 aa, canine distemper virus
MLPYQDKVGAFYKDNARANSTKLSLVTEGHGGRRPPYLLFVLLILLVGILALLAITGVRFHQVSTSNMEFSRLLKEDMEKSEAVHHQVIDVLTPLFKIIGDEIGLRLPQKLNEIKQFILQKTNFFNPNREFDFRDLHWCINPPSTVKVNFTNYCESIGIRKAIASAANPILLSALSGGRGDIFPPHRCSGATTSVGKVFPLSVSLSMSLISRTSEVINMLTAISDGVYGKTYLLVPDDIEREFDTREIRVFEIGFIKRWLNDMPLLQTTNYMVLPKNSKAKVCTIAVGELTLASLCVEESTVLLYHDSSGSQDGILVVTLGIFWATPMDHIEEVIPVAHPSMKKIHITNHRGFIKDSIATWMVPALASEKQEEQKGCLESACQRKTYPMCNQASWEPFGGRQLPSYGRLTLPLDASVDLQLNISFTYGPVILNGDGMDYYESPLLNSGWLTIPPKDGTISGLINKAGRGDQFTVLPHVLTFAPRESSGNCYLPIQTSQIRDRDVLIESNIVVLPTQSIRYVIATYDISRSDHAIVYYVYDPIRTISYTHPFRLTTKGRPDFLRIECFVWDDNLWCHQFYRFEADIANSTTSVENLVRIRFSCNR

SEQ ID NO: 9 - protein, 617 aa, measles virus
MSPQRDRINAFYKDNPHSKGSRIVINREHLMIDRPYVLLAVLFVMFLSLIGLLAIAGIRLHRAAIYTAEIHKSLSTNLDVTNSIEHQVKDVLTPLFKIIGDEVGLRTPQRFTDLVKFISDKIKFLNPDREYDFRDLTWCINPPERIKLNYDQYCADVAAEELMNALVNSTLLETRTTNQFLAVSKGNCSGPTTIRGQFSNMSLSLLDLYLSRGYNVSSIVTMTSQGMYGGTYLVEKPNLNSKGSELSQLSMYRVFEVGVIRNPGLGAPVFHMTNYFEQPISKDLSNCMVALGELKLAALCHGGDSITIPYQGSGKGVSFQLVKLGVWKSPTDMHSWVPLSTDDPVIDRLYLSSHRGVITDNQANWAVPTTRTDDKLRMETCFQQACKGKIQALCENLEWAPLKDSRIPSYGVLSVDLSLAAEPKIKIASGFGPLITHGSGMDLYKSNHNNVYWLTIPPMKNLALGVINTLEWIPRLKVSPNLFTVPIKEAGEDCHAPTYLPAEVDGDVKLSSNLVILPGQDLQYVLATYDTSRVEHAVVYYVYSPSRSFSYFYPFRLPIKGTPIELQVECFTWAQRLWCRHFCVLADSESGGHLTHSGMVGMEVSCTVNREDEANRR

SEQ ID NO: 10 - skipped

SEQ ID NO: 11 - DNA, 17 bp, synthetic construct
  misc_feature 1..17: note = construct sequence
  source 1..17: mol_type = other DNA
taatacgactcactata

SEQ ID NO: 12 - DNA, 68 bp, synthetic construct
  misc_feature 1..68: note = construct sequence
  source 1..68: mol_type = other DNA
taatacgactcactatagggagatgtttggtctgatgaggccgaaaggccgaaactccgtaaggagtc

SEQ ID NO: 13 - DNA, 70 bp, synthetic construct
  misc_feature 1..70: note = construct sequence
  source 1..70: mol_type = other DNA
taatacgactcactatagggagatttggtctgatgagtccgtgaggacgaaacggagtctagactccgtc

SEQ ID NO: 14 - DNA, 70 bp, synthetic construct; identical to SEQ ID NO: 13
  misc_feature 1..70: note = construct sequence
  source 1..70: mol_type = other DNA

SEQ ID NO: 15 - protein, 21 aa, synthetic construct
  REGION 1..21: note = construct sequence
KNLALGVINTLEWIPRFKVSP